European Patent Application EP 4 644 553 A1, published November 5, 2025. Title: NON-NUCLEIC ACID TARGET DETECTION METHOD BASED ON SPLIT CAS PROTEIN AND USE THEREOF. Applicant: SHANGHAI TOLO BIOTECHNOLOGY COMPANY LIMITED. The sequence listing filed with the application follows.

SEQUENCE LISTING (10 sequences)

SEQ ID NO: 1 - protein, 1228 aa, synthetic construct
MSKLEKFTNCYSLSKTLRFKAIPVGKTQENIDNKRLLVEDEKRAEDYKGVKKLLDRYYLSFINDVLHSIKLKNLNNYISLFRKKTRTEKENKELENLEINLRKEIAKAFKGNEGYKSLFKKDIIETILPEFLDDKDEIALVNSFNGFTTAFTGFFDNRENMFSEEAKSTSIAFRCINENLTRYISNMDIFEKVDAIFDKHEVQEIKEKILNSDYDVEDFFEGEFFNFVLTQEGIDVYNAIIGGFVTESGEKIKGLNEYINLYNQKTKQKLPKFKPLYKQVLSDRESLSFYGEGYTSDEEVLEVFRNTLNKNSEIFSSIKKLEKLFKNFDEYSSAGIFVKNGPAISTISKDIFGEWNVIRDKWNAEYDDIHLKKKAVVTEKYEDDRRKSFKKIGSFSLEQLQEYADADLSVVEKLKEIIIQKVDEIYKVYGSSEKLFDADFVLEKSLKKNDAVVAIMKDLLDSVKSFENYIKAFFGEGKETNRDESFYGDFVLAYDILLKVDHIYDAIRNYVTQKPYSKDKFKLYFQNPQFMGGWDKDKETDYRATILRYGSKYYLAIMDKKYAKCLQKIDKDDVNGNYEKINYKLLPGPNKMLPKVFFSKKWMAYYNPSEDIQKIYKNGTFKKGDMFNLNDCHKLIDFFKDSISRYPKWSNAYDFNFSETEKYKDIAGFYREVEEQGYKVSFESASKKEVDKLVEEGKLYMFQIYNKDFSDKSHGTPNLHTMYFKLLFDENNHGQIRLSGGAELFMRRASLKKEELVVHPANSPIANKNPDNPKKTTTLSYDVYKDKRFSEDQYELHIPIAINKCPKNIFKINTEVRVLLKHDDNPYVIGIDRGERNLLYIVVVDGKGNIVEQYSLNEIINNFNGIRIKTDYHSLLDKKEKERFEARQNWTSIENIKELKAGYISQVVHKICELVEKYDAVIALEDLNSGFKNSRVKVEKQVYQKFEKMLIDKLNYMVDKKSNPCATGGALKGYQITNKFESFKSMSTQNGFIFYIPAWLTSKIDPSTGFVNLLKTKYTSIADSKKFISSFDRIMYVPEEDLFEFALDYKNFSRTDADYIKKWKLYSYGNRIRIFRNPKKNNVFDWEEVCLTSAYKELFNKYGINYQQGDIRALLCEQSDKAFYSSFMALMSLMLQMRNSITGRTDVDFLISPVKNSDGIFYDSRNYEAQENAILPKNADANGAYNIARKVLWAIGQFKKAEDEKLDKVKIAISNKEWLEYAQTSVKH

SEQ ID NO: 2 - protein, 18 aa, synthetic construct
EFGGSGSSGGSGGSGGSG

SEQ ID NO: 3 - protein, 18 aa, synthetic construct
GGSGGSGGGSGSGSGGGT

SEQ ID NO: 4 - protein, 857 aa, synthetic construct
MSKLEKFTNCYSLSKTLRFKAIPVGKTQENIDNKRLLVEDEKRAEDYKGVKKLLDRYYLSFINDVLHSIKLKNLNNYISLFRKKTRTEKENKELENLEINLRKEIAKAFKGNEGYKSLFKKDIIETILPEFLDDKDEIALVNSFNGFTTAFTGFFDNRENMFSEEAKSTSIAFRCINENLTRYISNMDIFEKVDAIFDKHEVQEIKEKILNSDYDVEDFFEGEFFNFVLTQEGIDVYNAIIGGFVTESGEKIKGLNEYINLYNQKTKQKLPKFKPLYKQVLSDRESLSFYGEGYTSDEEVLEVFRNTLNKNSEIFSSIKKLEKLFKNFDEYSSAGIFVKNGPAISTISKDIFGEWNVIRDKWNAEYDDIHLKKKAVVTEKYEDDRRKSFKKIGSFSLEQLQEYADADLSVVEKLKEIIIQKVDEIYKVYGSSEKLFDADFVLEKSLKKNDAVVAIMKDLLDSVKSFENYIKAFFGEGKETNRDESFYGDFVLAYDILLKVDHIYDAIRNYVTQKPYSKDKFKLYFQNPQFMGGWDKDKETDYRATILRYGSKYYLAIMDKKYAKCLQKIDKDDVNGNYEKINYKLLPGPNKMLPKVFFSKKWMAYYNPSEDIQKIYKNGTFKKGDMFNLNDCHKLIDFFKDSISRYPKWSNAYDFNFSETEKYKDIAGFYREVEEQGYKVSFESASKKEVDKLVEEGKLYMFQIYNKDFSDKSHGTPNLHTMYFKLLFDEEFGGSGSSGGSGGSGGSGILWHEMWHEGLEEASRLYFGERNVKGMFEVLEPLHAMMERGPQTLKETSFNQAYGRDLMEAQEWCRKYMKSGNVKDLTQAWDLYYHVFRRISKGGSGGSGGGSGSGSGG

SEQ ID NO: 5 - protein, 641 aa, synthetic construct
MGGSGSSGGSGGSGGSGMGVQVETISPGDGRTFPKRGQTCVVHYTGMLEDGKKFDSSRDRNKPFKFMLGKQEVIRGWEEGVAQMSVGQRAKLTISPDYAYGATGHPGIIPPHATLVFDVELLKLEGGSGGSGGGSGSGSGGGTNNHGQIRLSGGAELFMRRASLKKEELVVHPANSPIANKNPDNPKKTTTLSYDVYKDKRFSEDQYELHIPIAINKCPKNIFKINTEVRVLLKHDDNPYVIGIDRGERNLLYIVVVDGKGNIVEQYSLNEIINNFNGIRIKTDYHSLLDKKEKERFEARQNWTSIENIKELKAGYISQVVHKICELVEKYDAVIALEDLNSGFKNSRVKVEKQVYQKFEKMLIDKLNYMVDKKSNPCATGGALKGYQITNKFESFKSMSTQNGFIFYIPAWLTSKIDPSTGFVNLLKTKYTSIADSKKFISSFDRIMYVPEEDLFEFALDYKNFSRTDADYIKKWKLYSYGNRIRIFRNPKKNNVFDWEEVCLTSAYKELFNKYGINYQQGDIRALLCEQSDKAFYSSFMALMSLMLQMRNSITGRTDVDFLISPVKNSDGIFYDSRNYEAQENAILPKNADANGAYNIARKVLWAIGQFKKAEDEKLDKVKIAISNKEWLEYAQTSVKH

SEQ ID NO: 6 - protein, 1062 aa, synthetic construct
MSKLEKFTNCYSLSKTLRFKAIPVGKTQENIDNKRLLVEDEKRAEDYKGVKKLLDRYYLSFINDVLHSIKLKNLNNYISLFRKKTRTEKENKELENLEINLRKEIAKAFKGNEGYKSLFKKDIIETILPEFLDDKDEIALVNSFNGFTTAFTGFFDNRENMFSEEAKSTSIAFRCINENLTRYISNMDIFEKVDAIFDKHEVQEIKEKILNSDYDVEDFFEGEFFNFVLTQEGIDVYNAIIGGFVTESGEKIKGLNEYINLYNQKTKQKLPKFKPLYKQVLSDRESLSFYGEGYTSDEEVLEVFRNTLNKNSEIFSSIKKLEKLFKNFDEYSSAGIFVKNGPAISTISKDIFGEWNVIRDKWNAEYDDIHLKKKAVVTEKYEDDRRKSFKKIGSFSLEQLQEYADADLSVVEKLKEIIIQKVDEIYKVYGSSEKLFDADFVLEKSLKKNDAVVAIMKDLLDSVKSFENYIKAFFGEGKETNRDESFYGDFVLAYDILLKVDHIYDAIRNYVTQKPYSKDKFKLYFQNPQFMGGWDKDKETDYRATILRYGSKYYLAIMDKKYAKCLQKIDKDDVNGNYEKINYKLLPGPNKMLPKVFFSKKWMAYYNPSEDIQKIYKNGTFKKGDMFNLNDCHKLIDFFKDSISRYPKWSNAYDFNFSETEKYKDIAGFYREVEEQGYKVSFESASKKEVDKLVEEGKLYMFQIYNKDFSDKSHGTPNLHTMYFKLLFDEEFGGSGSSGGSGGSGGSGVPLYGFTSICGRRPEMEAAVSTIPRFLQSSSGSMLDGRFDPQSAAHFFGVYDGHGGSQVANYCRERMHLALAEEIAKEKPMLCDGDTWLEKWKKALFNSFLRVDSEIESVAPETVGSTSVVAVVFPSHIFVANCGDSRAVLCRGKTALPLSVDHKPDREDEAARIEAAGGKVIQWNGARVFGVLAMSRSIGDRYLKPSIIPDPEVTAVKRVKEDDCLILASDGVWDVMTDEEACEMARKRILLWHKKNAVAGDASLLADERRKEGKDPAAMSAAEYLSKLAIQRGSKDNISVVVVDLKGGSGGSGGGSGSGSGG

SEQ ID NO: 7 - protein, 710 aa, synthetic construct
MGGSGSSGGSGGSGGSGTQDEFTQLSQSIAEFHTYQLGNGRCSSLLAQRIHAPPETVWSVVRRFDRPQIYKHFIKSCNVSEDFEMRVGCTRDVNVISGLPANTSRERLDLLDDDRRVTGFSITGGEHRLRNYKSVTTVHRFEKEEEEERIWTVVLESYVVDVPEGNSEEDTRLFADTVIRLNLQKLASITEAMNGGSGGSGGGSGSGSGGGTNNHGQIRLSGGAELFMRRASLKKEELVVHPANSPIANKNPDNPKKTTTLSYDVYKDKRFSEDQYELHIPIAINKCPKNIFKINTEVRVLLKHDDNPYVIGIDRGERNLLYIVVVDGKGNIVEQYSLNEIINNFNGIRIKTDYHSLLDKKEKERFEARQNWTSIENIKELKAGYISQVVHKICELVEKYDAVIALEDLNSGFKNSRVKVEKQVYQKFEKMLIDKLNYMVDKKSNPCATGGALKGYQITNKFESFKSMSTQNGFIFYIPAWLTSKIDPSTGFVNLLKTKYTSIADSKKFISSFDRIMYVPEEDLFEFALDYKNFSRTDADYIKKWKLYSYGNRIRIFRNPKKNNVFDWEEVCLTSAYKELFNKYGINYQQGDIRALLCEQSDKAFYSSFMALMSLMLQMRNSITGRTDVDFLISPVKNSDGIFYDSRNYEAQENAILPKNADANGAYNIARKVLWAIGQFKKAEDEKLDKVKIAISNKEWLEYAQTSVKH

SEQ ID NO: 8 - RNA, 42 nt, synthetic construct
  source 1..42: mol_type = other RNA
aatttctactcttgtagatttatcgcaactttctactgaatt

SEQ ID NO: 9 - DNA, 50 bp, synthetic construct
  source 1..50: mol_type = other DNA
ccgaattcagtagaaagttgcgataacaaaactggccgtcgttttacaac

SEQ ID NO: 10 - DNA, 50 bp, synthetic construct
  source 1..50: mol_type = other DNA
gttgtaaaacgacggccagttttgttatcgcaactttctactgaattcgg